European Patent Application EP 4 317 186 A1, published February 7, 2024. Title: NANOBODY TARGETING BCMA AND APPLICATION THEREOF. Applicant: ZHEJIANG NANOMAB TECHNOLOGY CENTER CO. LTD. The sequence listing filed with the application follows.

SEQUENCE LISTING (87 sequences)

SEQ ID NO: 1 - protein, 232 aa, Artificial Sequence
  Human IgG4 FC
EPKSADKTHTCPPCPAPELLGGPSVFLFPPKPKDTLMISRTPEVTCVVVDVSHEDPEVKFNWYVDGVEVHNAKTKPREEQYNSTYRVVSVLTVLHQDWLNGKEYKCKVSNKALPAPIEKTISKAKGQPREPQVYTLPPSREEMTKNQVSLTCLVKGFYPSDIAVEWESNGQPENNYKTTPPVLDSDGSFFLYSKLTVDKSRWQQGNVFSCSVMHEALHNHYTQKSLSLSPGK

SEQ ID NO: 2 - protein, 8 aa, Artificial Sequence
  NB-170 CDR1
EFIFSISA

SEQ ID NO: 3 - protein, 8 aa, Artificial Sequence
  NB-53/79/90/102/217/257/352/367 CDR1
GFTFSPSA

SEQ ID NO: 4 - protein, 8 aa, Artificial Sequence
  NB-29/36/51/65/71/84/100/122/192/265 CDR1
GFTFSSSA

SEQ ID NO: 5 - protein, 8 aa, Artificial Sequence
  NB-222 CDR1
GSIDRFYA

SEQ ID NO: 6 - protein, 8 aa, Artificial Sequence
  NB-34/67/82/216 CDR1
GSIFSIYA

SEQ ID NO: 7 - protein, 8 aa, Artificial Sequence
  NB-27/83 CDR1
GSISSIYA

SEQ ID NO: 8 - protein, 7 aa, Artificial Sequence
  NB-83 CDR2
ITSDNSA

SEQ ID NO: 9 - protein, 7 aa, Artificial Sequence
  NB-27 CDR2
ITSGGNT

SEQ ID NO: 10 - protein, 7 aa, Artificial Sequence
  NB-222 CDR2
ITSGGST

SEQ ID NO: 11 - protein, 7 aa, Artificial Sequence
  NB-67 CDR2
ITSGSST

SEQ ID NO: 12 - protein, 7 aa, Artificial Sequence
  NB-170 CDR2
ITTDGNS

SEQ ID NO: 13 - protein, 7 aa, Artificial Sequence
  NB-90 CDR2
IYGDGNA

SEQ ID NO: 14 - protein, 7 aa, Artificial Sequence
  NB-79 CDR2
IYGDGRA

SEQ ID NO: 15 - protein, 7 aa, Artificial Sequence
  NB-352 CDR2
IYGDGRP

SEQ ID NO: 16 - protein, 7 aa, Artificial Sequence
  NB-367 CDR2
IYGEGST

SEQ ID NO: 17 - protein, 7 aa, Artificial Sequence
  NB-1/102 CDR2
IYPDGRT

SEQ ID NO: 18 - protein, 7 aa, Artificial Sequence
  NB-51 CDR2
IYPDGSA

SEQ ID NO: 19 - protein, 7 aa, Artificial Sequence
  NB-36/53 CDR2
IYPDGST

SEQ ID NO: 20 - protein, 7 aa, Artificial Sequence
  NB-84/100 CDR2
IYPDGTA

SEQ ID NO: 21 - protein, 7 aa, Artificial Sequence
  NB-71 CDR2
IYPDGTP

SEQ ID NO: 22 - protein, 7 aa, Artificial Sequence
  NB-257 CDR2
IYSDGRA

SEQ ID NO: 23 - protein, 7 aa, Artificial Sequence
  NB-29/65/122/192/217/265 CDR2
IYSDGST

SEQ ID NO: 24 - protein, 7 aa, Artificial Sequence
  NB-216 CDR2
VTSAGNT

SEQ ID NO: 25 - protein, 7 aa, Artificial Sequence
  NB-34 CDR2
VTSEGGT

SEQ ID NO: 26 - protein, 7 aa, Artificial Sequence
  NB-82 CDR2
VTTEGST

SEQ ID NO: 27 - protein, 17 aa, Artificial Sequence
  NB-192 CDR3
AIGAPDPFDYSGWRRHL

SEQ ID NO: 28 - protein, 17 aa, Artificial Sequence
  NB-122 CDR3
AIGAPDPFDYSGWRRNL

SEQ ID NO: 29 - protein, 19 aa, Artificial Sequence
  NB-65 CDR3
AIGDVRGRWDSRPRHEWTY

SEQ ID NO: 30 - protein, 13 aa, Artificial Sequence
  NB-53 CDR3
AIGLAPGYRDPNL

SEQ ID NO: 31 - protein, 15 aa, Artificial Sequence
  NB-84 CDR3
AIGRWYDQRKKEPGL

SEQ ID NO: 32 - protein, 15 aa, Artificial Sequence
  NB-90 CDR3
AIGRWYEGRKKEEGL

SEQ ID NO: 33 - protein, 13 aa, Artificial Sequence
  NB-29 CDR3
AVGAPLVYAAYRP

SEQ ID NO: 34 - protein, 13 aa, Artificial Sequence
  NB-265 CDR3
AVGAPLVYASYRP

SEQ ID NO: 35 - protein, 17 aa, Artificial Sequence
  NB-217 CDR3
AVGIVVPYSEDAWYSTL

SEQ ID NO: 36 - protein, 15 aa, Artificial Sequence
  NB-352 CDR3
AVGLWYEKREKEKDL

SEQ ID NO: 37 - protein, 15 aa, Artificial Sequence
  NB-100 CDR3
AVGRWYEQRKKEPGL

SEQ ID NO: 38 - protein, 14 aa, Artificial Sequence
  NB-170 CDR3
DVAPWGYHAPEVGS

SEQ ID NO: 39 - protein, 15 aa, Artificial Sequence
  NB-79 CDR3
GIGRWYDQREKEKDL

SEQ ID NO: 40 - protein, 15 aa, Artificial Sequence
  NB-257 CDR3
GIGRWYEKREKEKGF

SEQ ID NO: 41 - protein, 15 aa, Artificial Sequence
  NB-102 CDR3
GIGRWYENREKEKDL

SEQ ID NO: 42 - protein, 15 aa, Artificial Sequence
  NB-367 CDR3
GVGRWYEGRQYEHDY

SEQ ID NO: 43 - protein, 15 aa, Artificial Sequence
  NB-222 CDR3
NAAPWGDYTAHDFAS

SEQ ID NO: 44 - protein, 16 aa, Artificial Sequence
  NB-34 CDR3
NAAPWGSYHPQSDIFS

SEQ ID NO: 45 - protein, 16 aa, Artificial Sequence
  NB-82 CDR3
NAAPWGSYHPQTDIVS

SEQ ID NO: 46 - protein, 17 aa, Artificial Sequence
  NB-27 CDR3
NAAPWGSYSPGPGDIAS

SEQ ID NO: 47 - protein, 15 aa, Artificial Sequence
  NB-67 CDR3
NPAPWGDYTATDFHS

SEQ ID NO: 48 - protein, 17 aa, Artificial Sequence
  NB-216 CDR3
NSAPWGSYSPGPADVSS

SEQ ID NO: 49 - protein, 17 aa, Artificial Sequence
  NB-83 CDR3
NVAPWGSYSPGPADIAS

SEQ ID NO: 50 - protein, 13 aa, Artificial Sequence
  NB-51 CDR3
QVGRYVSGVDYQP

SEQ ID NO: 51 - protein, 14 aa, Artificial Sequence
  NB-36 CDR3
VIGRRGYAMGDRRL

SEQ ID NO: 52 - protein, 14 aa, Artificial Sequence
  NB-71 CDR3
VVGRRGYAMGDRAL

SEQ ID NO: 53 - protein, 123 aa, Artificial Sequence
  NB-27 antibody amino acid sequence
EVQLVESGGGLVQPGGSLRLSCAASGSISSIYAMGWYRQAPGKLRGLVAAITSGGNTFYADSVKGRFTISRDNAKNTVYLQMNSLKPEDTAVYDCNAAPWGSYSPGPGDIASWGQGTQVTVSS

SEQ ID NO: 54 - protein, 119 aa, Artificial Sequence
  NB-29 antibody amino acid sequence
EVQLVESGGGLVQPGESLRLSCAASGFTFSSSAMSWARQAPGKGLEWVSGIYSDGSTYYADSVKGRFTISRDNAKNTVYLQMNSLKPEDTAVYLCAVGAPLVYAAYRPWGQGTQVTVSS

SEQ ID NO: 55 - protein, 122 aa, Artificial Sequence
  NB-34 antibody amino acid sequence
EVQLVESGGGLVQPGGSLRLSCAASGSIFSIYAMGWYRQAPGKQRELVAAVTSEGGTFYRDSVKGRFTISRDNAKNTVYLQMNSLKPEDTAVYQCNAAPWGSYHPQSDIFSWGQGTQVTVSS

SEQ ID NO: 56 - protein, 120 aa, Artificial Sequence
  NB-36 antibody amino acid sequence
QVQLVESGGGLVQPGGSLRLSCAASGFTFSSSAMSWARRPPGKGLEWVSDIYPDGSTTYADSMKGRFTISRDNAKNTVYLEIYSLKPEDTAVYYCVIGRRGYAMGDRRLRGQGTQVTVSS

SEQ ID NO: 57 - protein, 119 aa, Artificial Sequence
  NB-51 antibody amino acid sequence
QVQLVESGGGLAQPGGSLRLSCAASGFTFSSSAMSWARQAPGKGLEWVSDIYPDGSAYYADSMKGRFTISRDNAKNTVYLQMDSLKPEDTAVYHCQVGRYVSGVDYQPRGQGTQVTVSS

SEQ ID NO: 58 - protein, 119 aa, Artificial Sequence
  NB-53 antibody amino acid sequence
QVQLVESGGGLVQPGGSLRLSCAASGFTFSPSAMSWARQAPGKGLEWVSSIYPDGSTLYADSMKGRFTISRDNAKNTVSLQMNSLKPEDTAVYYCAIGLAPGYRDPNLRGQGTQVTVSS

SEQ ID NO: 59 - protein, 125 aa, Artificial Sequence
  NB-65 antibody amino acid sequence
QVQLVESGGGLVQPGGSLRLSCAASGFTFSSSAMSWARQAPGKELEWVSAIYSDGSTYYADSVKGRFTISRDNAKNTIYLQMNSLKPEDTANYICAIGDVRGRWDSRPRHEWTYWGQGTQVTVSS

SEQ ID NO: 60 - protein, 121 aa, Artificial Sequence
  NB-67 antibody amino acid sequence
QVQLVESGGGLVQPGGSLRLSCTASGSIFSIYAMGWYRQAPGKPRELVAAITSGSSTFYRDSVKGRFTISRDNAKNTVYLRMNSLKPEDTAVYYCNPAPWGDYTATDFHSWGQGTQVTVSS

SEQ ID NO: 61 - protein, 120 aa, Artificial Sequence
  NB-71 antibody amino acid sequence
EVQLVESGGGLVQPGGSLRLSCAASGFTFSSSAMSWARQAPGKGLEWVSDIYPDGTPTYADSMEGRFTISRDNAKNTVHLQIDSLKPEDTAVYYCVVGRRGYAMGDRALRGQGTQVTVSS

SEQ ID NO: 62 - protein, 121 aa, Artificial Sequence
  NB-79 antibody amino acid sequence
EVQLVESGGGSVQPGGSLRLSCAASGFTFSPSAMSWARQAPGKGFEWVSSIYGDGRAYYADSMKGRFTISRDNAKHTVYLQMNSLKPEDTALYYCGIGRWYDQREKEKDLWGQGTQVTVSS

SEQ ID NO: 63 - protein, 122 aa, Artificial Sequence
  NB-82 antibody amino acid sequence
EVQLVESGGGLVQPGGSLRLSCAASGSIFSIYAMGWYRQAPGKPRELVAAVTTEGSTFYRDSVKGRFTISRDNAKNAVYLQMNSLKPEDTAVYQCNAAPWGSYHPQTDIVSWGQGTQVTVSS

SEQ ID NO: 64 - protein, 123 aa, Artificial Sequence
  NB-83 antibody amino acid sequence
QVQLVESGGGLVQPGGSLRLSCAASGSISSIYAMGWYRQAPGKQRELVAAITSDNSAFYRDSVKGRFTISRDNAKNTVYLQMDSLKVEDTAVYDCNVAPWGSYSPGPADIASWGQGTQVTVSS

SEQ ID NO: 65 - protein, 121 aa, Artificial Sequence
  NB-84 antibody amino acid sequence
QVQLVESGGGLVQPGGSLRLSCAASGFTFSSSAMSWARQAPGKGLEWVSSIYPDGTAYYADSMKGRFAISRDNARNTVYLQMNSLKPEDTALYQCAIGRWYDQRKKEPGLWGQGTQVTISS

SEQ ID NO: 66 - protein, 121 aa, Artificial Sequence
  NB-90 antibody amino acid sequence
QVQLVESGGGLVQPGESLRLSCAASGFTFSPSAMSWARQAPGKGLEWVSSIYGDGNAYYSDSMKGRFTISRDNAKNTVYLQMNSLKPEDTALYYCAIGRWYEGRKKEEGLWGQGTQVTVAS

SEQ ID NO: 67 - protein, 121 aa, Artificial Sequence
  NB-100 antibody amino acid sequence
QVQLVESGGGLVQPGGSLRLSCAASGFTFSSSAMSWARQAPGKGLEWVSSIYPDGTAYYADSMKGRFAISRDNARNTVYLQMNSLKPEDTALYQCAVGRWYEQRKKEPGLWGQGTQVTISS

SEQ ID NO: 68 - protein, 121 aa, Artificial Sequence
  NB-102 antibody amino acid sequence
QVQLVESGGDLVQPGGSLRLSCAASGFTFSPSAMSWARQAPGKGFEWVSTIYPDGRTYYSDSMKGRFTISRDNAKNTVYLQMHSLKPEDTALYYCGIGRWYENREKEKDLWGQGTQVTVSS

SEQ ID NO: 69 - protein, 123 aa, Artificial Sequence
  NB-122 antibody amino acid sequence
QVQLVESGGGLVQPGGSLRLSCAASGFTFSSSAMSWARQAPGMGLERVSSIYSDGSTYYPDSMKGRFTISRDNAKNTVYLQMNSLKPEDTAVYICAIGAPDPFDYSGWRRNLLGQGTQVTVSS

SEQ ID NO: 70 - protein, 120 aa, Artificial Sequence
  NB-170 antibody amino acid sequence
QVQLVESGGGLVQPGGSLRLSCAASEFIFSISAMSWYRQAPGKVLELVSDITTDGNSFYADSMKGRFTISRDNAKNTMYLQMNILKSEDTAAYDCDVAPWGYHAPEVGSWGQGTLVTVSS

SEQ ID NO: 71 - protein, 123 aa, Artificial Sequence
  NB-192 antibody amino acid sequence
QVQLVESGGGLVQPGGSLRLSCAASGFTFSSSAMSWARQAPGKGLERVSSIYSDGSTYYSDSMKGRFTISRDNAKNTVYLQMNSLKPEDTAVYYCAIGAPDPFDYSGWRRHLLGQGTLVTVSS

SEQ ID NO: 72 - protein, 123 aa, Artificial Sequence
  NB-216 antibody amino acid sequence
QVQLVESGGGLVQPGGSLRLTCAASGSIFSIYAMGWYRQAPGKQRELVAAVTSAGNTFYRDSVKGRFTISRDNAKSTVYLQMNSLKPEDTAVYDCNSAPWGSYSPGPADVSSWGQGTLVTVSS

SEQ ID NO: 73 - protein, 123 aa, Artificial Sequence
  NB-217 antibody amino acid sequence
EVQLVESGGGTVQPGGSLRLSCVASGFTFSPSAMSWVRQAPGKGLEWVSGIYSDGSTRYADSVKGRFTISRDNVKNTVYLQMNSLNPEDTAVYYCAVGIVVPYSEDAWYSTLRGQGTQVTVSS

SEQ ID NO: 74 - protein, 121 aa, Artificial Sequence
  NB-222 antibody amino acid sequence
QVQLVESGGGLVQPGGSLRLSCAASGSIDRFYAMGWYRQAPGKSRTLVTAITSGGSTYYADSVKGRFTISRDNAKNMLYLQMNSLKPEDTAVYYCNAAPWGDYTAHDFASWGQGTQVTVSS

SEQ ID NO: 75 - protein, 121 aa, Artificial Sequence
  NB-257 antibody amino acid sequence
EVQLVESGGGLVQPGGSLRLSCAASGFTFSPSAMSWARQAPGKGFEWVSSIYSDGRAYYADTMKGRFTISRDNAKNTVYLQMNSLRPEDTALYYCGIGRWYEKREKEKGFWGQGTQVTVSS

SEQ ID NO: 76 - protein, 119 aa, Artificial Sequence
  NB-265 antibody amino acid sequence
EVQLVESGGGLVQPGESLRLSCAASGFTFSSSAMSWARQAPGKGLEWVSGIYSDGSTYYADSVKGRFTISRDNAKNTVYLQMNSLKPEDTAVYKCAVGAPLVYASYRPWGQGTLVTVSS

SEQ ID NO: 77 - protein, 121 aa, Artificial Sequence
  NB-352 antibody amino acid sequence
QVQLVESGGGLVQPGGSLRLSCAASGFTFSPSAMSWARQAPGKGLEWVASIYGDGRPYYADSMKGRFTISRDNAKNTVYLQMNSLKPEDTALYYCAVGLWYEKREKEKDLWGQGTQVTVSS

SEQ ID NO: 78 - protein, 121 aa, Artificial Sequence
  NB-367 antibody amino acid sequence
QVQLVESGGGLVQPGGSLRLSCAASGFTFSPSAMSWARRAPGKGLEWVSSIYGEGSTVYADSMKDRFTISRDNAKNTVYLQMNSLKPEDTAVYYCGVGRWYEGRQYEHDYWGQGTLVTVSS

SEQ ID NO: 79 - protein, 8 aa, Artificial Sequence
  NB-1 CDR1
GFTFRSSA

SEQ ID NO: 80 - protein, 13 aa, Artificial Sequence
  NB-1 CDR3
QVGRYVSGVYYQP

SEQ ID NO: 81 - protein, 246 aa, Artificial Sequence
  BMK1
DIVLTQSPASLAVSLGKRATINCRASESVSVIGAHLIHWYQQKPGQPPKLLIYLASNLETGVPARFSGSGSGTDFTLTISSLQAEDAAIYYCLQSRIFPRTFGGGTKLEIKGSTSGSGKPGSGEGSTKGQVQLVQSGSELKKPGASVKVSCKASGYTFTDYSINWVRQAPGQGLEWMGWINTETREPAYAYDFRGRFVFSLDTSVSTAYLQISSLKAEDTAVYYCARDYSYAMDYWGQGTLVTVSS

SEQ ID NO: 82 - protein, 243 aa, Artificial Sequence
  BMK3
QVQLVQSGAEVKKPGSSVKVSCKASGGTFSNYWMHWVRQAPGQGLEWMGATYRGHSDTYYNQKFKGRVTITADKSTSTAYMELSSLRSEDTAVYYCARGAIYDGYDVLDNWGQGTLVTVSSGGGGSGGGGSGGGGSDIQMTQSPSSLSASVGDRVTITCSASQDISNYLNWYQQKPGKAPKLLIYYTSNLHSGVPSRFSGSGSGTDFTLTISSLQPEDFATYYCQQYRKLPWTFGQGTKLEIK

SEQ ID NO: 83 - protein, 119 aa, Artificial Sequence
  NB-1 antibody amino acid sequence
EVQLVESGGGLVQPGGSLRLSCAASGFTFRSSAMSWARQAPGKGLEWVSDIYPDGRTDYADSIKGRFTMSRDNAKNTVYLLMDSLKPEDTAVYHCQVGRYVSGVYYQPRGQGTQVTVSS

SEQ ID NO: 84 - DNA, 24 bp, Artificial Sequence
  upstream primer 1
gtcctggctgctcttctacaaggc

SEQ ID NO: 85 - DNA, 23 bp, Artificial Sequence
  downstream primer 1
ggtacgtgctgttgaactgttcc

SEQ ID NO: 86 - DNA, 29 bp, Artificial Sequence
  upstream primer 2
gatgtgcagctgcaggagtctggrggagg

SEQ ID NO: 87 - DNA, 35 bp, Artificial Sequence
  downstream primer 2
ggactagtgcggccgctggagacggtgacctgggt